European Patent Application EP 4 512 899 A1, published February 26, 2025. Title: ANGPTL4 ASO compositions for treatment of atherosclerosis in humans. Applicant: LIPIGON PHARMACEUTICALS AB. The sequence listing filed with the application follows.

SEQUENCE LISTING (252 sequences)

SEQ ID NO: 1 - DNA, 1905 bp, Homo sapiens
  source 1..1905: mol_type = genomic DNA
ataaaaaccgtcctcgggcgcggcggggagaagccgagctgagcggatcctcacacgactgtgatccgattctttccagcggcttctgcaaccaagcgggtcttacccccggtcctccgcgtctccagtcctcgcacctggaaccccaacgtccccgagagtccccgaatccccgctcccaggctacctaagaggatgagcggtgctccgacggccggggcagccctgatgctctgcgccgccaccgccgtgctactgagcgctcagggcggacccgtgcagtccaagtcgccgcgctttgcgtcctgggacgagatgaatgtcctggcgcacggactcctgcagctcggccaggggctgcgcgaacacgcggagcgcacccgcagtcagctgagcgcgctggagcggcgcctgagcgcgtgcgggtccgcctgtcagggaaccgaggggtccaccgacctcccgttagcccctgagagccgggtggaccctgaggtccttcacagcctgcagacacaactcaaggctcagaacagcaggatccagcaactcttccacaaggtggcccagcagcagcggcacctggagaagcagcacctgcgaattcagcatctgcaaagccagtttggcctcctggaccacaagcacctagaccatgaggtggccaagcctgcccgaagaaagaggctgcccgagatggcccagccagttgacccggctcacaatgtcagccgcctgcaccggctgcccagggattgccaggagctgttccaggttggggagaggcagagtggactatttgaaatccagcctcaggggtctccgccatttttggtgaactgcaagatgacctcagatggaggctggacagtaattcagaggcgccacgatggctcagtggacttcaaccggccctgggaagcctacaaggcggggtttggggatccccacggcgagttctggctgggtctggagaaggtgcatagcatcacgggggaccgcaacagccgcctggccgtgcagctgcgggactgggatggcaacgccgagttgctgcagttctccgtgcacctgggtggcgaggacacggcctatagcctgcagctcactgcacccgtggccggccagctgggcgccaccaccgtcccacccagcggcctctccgtacccttctccacttgggaccaggatcacgacctccgcagggacaagaactgcgccaagagcctctctggaggctggtggtttggcacctgcagccattccaacctcaacggccagtacttccgctccatcccacagcagcggcagaagcttaagaagggaatcttctggaagacctggcggggccgctactacccgctgcaggccaccaccatgttgatccagcccatggcagcagaggcagcctcctagcgtcctggctgggcctggtcccaggcccacgaaagacggtgactcttggctctgcccgaggatgtggccgttccctgcctgggcaggggctccaaggaggggccatctggaaacttgtggacagagaagaagaccacgactggagaagccccctttctgagtgcaggggggctgcatgcgttgcctcctgagatcgaggctgcaggatatgctcagactctagaggcgtggaccaaggggcatggagcttcactccttgctggccagggagttggggactcagagggaccacttggggccagccagactggcctcaatggcggactcagtcacattgactgacggggaccagggcttgtgtgggtcgagagcgccctcatggtgctggtgctgttgtgtgtaggtcccctggggacacaagcaggcgccaatggtatctgggcggagctcacagagttcttggaataaaagcaacctcagaacactttg

SEQ ID NO: 2 - DNA, 10223 bp, Homo sapiens
  source 1..10223: mol_type = genomic DNA
ggggagaagccgagctgagcggatcctcacacgactgtgatccgattctttccagcggcttctgcaaccaagcgggtcttacccccggtcctccgcgtctccagtcctcgcacctggaaccccaacgtccccgagagtccccgaatccccgctcccaggctacctaagaggatgagcggtgctccgacggccggggcagccctgatgctctgcgccgccaccgccgtgctactgagcgctcagggcggacccgtgcagtccaagtcgccgcgctttgcgtcctgggacgagatgaatgtcctggcgcacggactcctgcagctcggccaggggctgcgcgaacacgcggagcgcacccgcagtcagctgagcgcgctggagcggcgcctgagcgcgtgcgggtccgcctgtcagggaaccgaggggtccaccgacctcccgttagcccctgagagccgggtggaccctgaggtccttcacagcctgcaggtacgtgtccccagggctggttctccgcgcccctagtggctctcctggcttggaagggtatggacaggagtggggcgtgggggcggggtgcgcaactgtggctccctgggcttccctgcgtcaagggatgggctccccccttaggaagccgaggagggaggttcgctcaaggccaggaattcaagaccacctaaagcaaaatagcgagacccccgtctcttctacacacacacacacacacacacaaaataaataaaataaaataaaataaatataaaattaaaaaacgaccgggcgcagtggctcacggagcctccacctgctgtcgagactagcctggccaacatggagaaacctcgtctctactaaaaatacaaaaaattagcctggcatggtgtgcatgcctgtaatcccagctacttgggaggctgaggcaggagaatctcttgaacccgggaggcagaggttgcagtgagccgagatcgcagcactgcactccagcctgggcaacagagtgagactcctcaaaaaaataatagcgataaaataaaaataaagccaggtgcggtgactcacgcttgtagtcccagcactttgggagggcgaggccagtggatcacctgaggtcaggagttcaagaccagcctgaccaacacagtgaaaccccgtctctactaaaaatacaaaaattagctgggtgtggtggtgggcgcctgtaatcccagctactggggaggctgaggcaggagaacctcttgaacccgggaggcggaggttgcagtgagccgggatcatgccattgcactccagcctgggcgacagagctcgactccatctcaaaataataataataataaataaaataaaatacaaatacaaaaattagccaggtgtggtggcagctacttgggaggctgagacacaagaatcacttgagtctgggaggcagaggttgcagtgagccaagattgcgccactgcactccaacctgggtgacagagcgagactctgtctgaaaaaataaaaaataagccaggcatagagctgcatgactgtagtcccagctacacaggaggctgaaaacaggaggatcgcctgaccccaggagttggaggctgcagtgagctgtgacagcaccactgcactccagcctgggcgagagaacgagaccccgtcattgggaaaaaaaagaaaaaagaaagactcccttgcctggcctcagcggatggagatttggaaggatggatgagtggatgaattaagaggttggggtaggcaagctgggtcctcaccaaggttttcacccctccccagacacaactcaaggctcagaacagcaggatccagcaactcttccacaaggtggcccagcagcagcggcacctggagaagcagcacctgcgaattcagcatctgcaaagccaggtaaccctaggatcaagggagaaaaggtccctctgatagctggaccccaggttgagagggaggtggtgagaactggacgtgtggctggggacgtggggccaggcaggacctgacaccctcctcccgtcccatcctagtttggcctcctggaccacaagcacctagaccatgaggtggccaagcctgcccgaagaaagaggctgcccgagatggcccagccagttgacccggctcacaatgtcagccgcctgcaccgtgagtgtctgcccctcgatgctctccggtggccacccctaccccgccacttgccattgctggtcctctccttgtcaggtccaccttaaggagaagatgtcctggcctggagtccctgagggctcaccagtctctgggtcaaagctgatgggagcacctccttcctcagccctgacctggcccagccaggccacccaacccttctcctctgcaagccagtgggctgtccctgaagccctgctgatcactgattggaacagaggtggagaaagaggtcttgagggacttgagctgcaggggtgctggagaaggtagaaatggggttcggggtgccatcctgaaggttagaaccttctaggggagggtgtcatggaggagggggtgccaggtagtagtgtttgtagatttgggccctccacaatgtcttggggtatgtgggaattagggctgggaacccccagctcccagaccagaaacactcttgtatcttacaaatccaatgctccaggtccctgacccctcttcctccttcctctcttgttctcctcctccctccccgcccccgccggccccctccccaccgcagaaagtgggcttttgctgccaccacaagttgtaggtgctttattcccaaatctccgttcatctcgaaccacagcatgtccacgtgtgtccgatgcagactcgcggttctctaagttcacggccccacacggtttctctgtggtcctcatccttccctgcatctgtggctgtccacagccaactgggtgaaagtttggatccccctctcacaccctagggtcagtggcaggcttccagcactgtagacctgagggttctctcctccccaagctcccgctccttcccacctccgtgctgcccgcccccaaccccgccaggctagcatctcagcgtggtcagggtcctgtccaccctcccaaagccaccatcccaggatgaggggcttctggagggtgacgggggaaggcacaagtcctggctgggaaatgcggtggaagggggcaggggttctgtgggttcgggactcccagactcttggctcaggcccgccaagtaggagaaagttcagagctgggaaggcgaacagctggcattcatggaagccacactggtggtttggccgcgtgcccatccttactggatgggaggaaagtaggggaaaggggagatgcctgaggggccggaaagcgtcttcctggtcactctgggcccgcccccacccccaccgtgcagactcatttcgacctttcccctacttttccggctgggctgggggcggttcctcccagtctggagcgtctgagcctccagacgtgctcaacgccatcctcccctcctccctccctctttctttcctcaaccctgcctcctctccctctaggagctgggaccccaggcagagcctctgagatgctcctgctcagcacagttcttcccgttctggacctgctgcctcattcattcattcattcattcatttgtcaagactgttttgtttgctttttgagacggagtctcgctctgttgtccaggctggagtgcagtggcgcaatctcagctcactgcaacctctgcctcccactgggttcaagtgattctcctgcctcagcctctcaagtagatgggattataggcgcctaccgccaccacgcccagctaatttttattcatttatcaagtcttttttttttttgagacagagtctcactctgtcacccaggttggagtgcaatggttcaacctcagctgactgcaacctctgcctcccgggttcaagtgattctcctgcctctgcctcctaaggagctgggattactggcgtccaccatcacacccagctaatctttgtatgttttactagagatggggtttggccatgttgaccaggctggtctcaaactcctgaccgatccgcccgcctcccaaagtgctggattacaggcatgaaccactgcgcccggcccattcctcaagtctttattgagcagctgctatgcgctggggcctgcgtggatgctggtgccaggctgtgggcagagctgctccttgtccccagcctcatggagcctccattgagtcagaggagagaccattagatgacctcagtgtccaggagtgggaagtccttgctcaattcccatttggggtgttctggcctggtctgggggtgaggcaaggcagggtgtccttccagaagctgggacccagagagagaagtgaggaaagagagtcccgccgggcgcagtggttcacacctgtaatcccagcactttgggaggccaaggctggcggatcacgaggtcaggagatcgagaccagtctggccaacatggtgaaacccccgtctctacaaataatgcaaaaactagtcgggcgtggtggcacatgcctgtagtcccagctgctccggaggctgcggcagaattgcttgaacctgggaggcggaggttgcagtgagccaagattgcgccactgcactccagcctggcgacagagcgagactccgtatcaaaaaacaaaacaaaaaaagagagtcccaggcagggggaacagcatgtgcaaagtccctgtggcaggacggtgtgtggtacaagggtgggaagaaagcctgtgtgccagagagggtgtgggtacagcatggcaggaggaggatgggcacgggggctggtcctccaggtgccttgtggaccatgctgaggaaggacatagggagccatggaagaggttaggcagatggcagagaggtggtcatgagataagatttgccttttacttccctggtcatccactgttaagcccccagatatgcctggctcctgagaccccccccaggggctgccctcctgtttcaagtctccactttatctcccttcagggctgcccagggattgccaggagctgttccaggttggggagaggcagagtggactatttgaaatccagcctcaggggtctccgccatttttggtgaactgcaagatgacctcaggtagggtgtgttagtccaccaggggcccctctccccataggccctgttgtctttctttaaattgaaaacaaaacaaaacaaaaaaattaaaggcagggtcttgctatgttgcccaagctggtctttttttttttttttttttttgagatggagttttgctcttggagctggagtgcaatgccacgatctcagctcactgaaacctccgcctcccgggttcaagcaattctccagcgtcagcctccccagtagctgagactacaggtgcgagcaaccacacccagctaatttttgtatttttagtagagactgggtttcaccatgttggtctggctggtctcaaactcctgacctcaaatgatttgccgactttggcctcccaaaatgctgggattataggcattagccactgctcctggcctcttttctttaaaatgcagcccttgtctgggtgtagtggctcatatctgtaatcccgacactttgggaggcctatcatgaggatcacttgagcccagaagttcgagaccagcctggacaacatagtgagagctcatctttacaaaaaattttgtaaaagtaaaaaaaaaggccaagtgcagtggctcacacctgtaatcccagcactttgggaggttgaggcagacagatcacgaggtcaggagttcgagaccagcctgaccaacatggtgaaaccccgtctctactaaaaatacaaaaattagccgggcatggtggtgtgcacctgtaatcccagctactcaggtggctgaggcaggagaatctcttgaacctgggaggcagaggttgcagtgagctgagatgacgccaccgcactccagcctgggcgacagagcgagactccgtccccccatcaaaaaaataaaaaagagaaaataaaataaaataaaataaaattcagcccttgctgggcatggtggcacatgcctgtagtcccagctactcgggaggccaaggcaggagggtcacttcagcccaggagttaaaggctgccgtgagccgtgatcacacctgtgaatagccaccgcactccaacctgggcaacacaacaaaacctcgtttctaaaaaaaaacaaaggctgagcacggtggcttacacctgaaatgccagcactttgggaggctgaggcgggcaaatcacttgaggtcagaagttcaagaccagcctggccaacatggtgaaaccctatctctaccaacataaacattagccgggcgtgcctgtgattccagctgcttgtggggctgaagcacaagaatcgcttgagccccgaaggcagaggttgcagtgagctgagattgcggcactgcgatccagcctgggcaacagagtgagactccatctctaaaaaaaaaaaaaaaaaaaaagaaagcttttttttccactgagaagtcctttccattacaagaggttacaacacggggttttacccagttcagctggcccagagaggctttgcagatttccactgcctactccctcccacactcagtccctgctgggttcttgggacaaagatcttcccaaggccagcccataatattcctccctctgacccaccctcctcgagtcctccagggatgagtgagggagctgctgtcttcctgggtttggagggggtttggtgcttggcagccagatgagggagtggggtcgtctgtgaagagggacttcctggtgaccttgtacctttctgggcagatggaggctggacagtaattcagaggcgccacgatggctcagtggacttcaaccggccctgggaagcctacaaggcggggtttggggatccccacggtaggtgtttctagtggggacagaggcaggggaggaagagggaccctcagaagtggccctgcctcatggagtggcctctcccactccaggcgagttctggctgggtctggagaaggtgcatagcatcacgggggaccgcaacagccgcctggccgtgcagctgcgggactgggatggcaacgccgagttgctgcagttctccgtgcacctgggtggcgaggacacggcctatagcctgcagctcactgcacccgtggccggccagctgggcgccaccaccgtcccacccagcggcctctccgtacccttctccacttgggaccaggatcacgacctccgcagggacaagaactgcgccaagagcctctctggtgagcaggccctgccatgccacacccagccagcagcttccctccttatctttctgctgctctgtcctgccttcaaccccacattgcatctgtttcctgcccccacctcttccttacatgccgtgtgtgtgattgggccactaacttagcctatctggcctcagttttcccatcctgaaaagggtcttgaccgtctttacttttatttacttatgtgtttgtttatttatttatttatgtatttattttttgagacggagtctcactttgtcacccaggctggagtgctttgtggcacgatcttggctcactgcaagctccacctcctgagttcacaccattctcctgcctcagcctcccgagtagctgggactataggtgcccaccaccacgcctggctaatttttttgtatttttagtagagatggggtttcaccgtgttagccaggatggtctcgatctcctgacctcgtgatctgcctgcctcagcctcccaaagtgctgggattacaggcgtgagccaccgcgcccggcctacttatttattttttgagacagagtcccgctgtgtctcccaggctggagtgcaagtgacgtgatcttggctcactgcagcctccgcctcctgggttcaagtgattctcctgcctcagcctcctgagtagctgggattacaggttcccgccaccatgcacagataattgttttgtatttttagtagagacggggtttcaccatgttggccagggtggtcttgaactcctgacctcaagtgatctgcccacctcggcctcccaaagtgttgggattacaggcgtgagccacaatacccggccacaaacatctttataatggtgctccacaggattctttttttttttttttttttgaaacagggtctcactctgttgcctaagctggagtgcagtggtgcgatctcggctcactgcaacctccacctcccgggttcaagcaattctcaaaaaaaaaaaaaaattaggcacggtggctcacacttgcaatcccagcactttgggaggctgaagcgagtggatcacttgagcccaggagaccaatctgagcaacagggcgaaatcctgtctcaattaaaaatacaaaaaactagctgggcatggtggtgcctgcctgtgttcccatctacttgggaggctgagttgggaggatctcttgagcctaggagataaggctgcagtgagctgagactgcgccactgcactcaagcctgggtgacagagtgagacccctgcctcaaaagaaaaagaaaaaatgcaggcatggtggctcacacctgtggtcccagctacttgggaggcccaggtacaagaatcacttgagcccgtaaggttgacgctgcattgagccatcaccacaccactgcactccagcctgggcaatggagccaggccctgtctcaaaaaaaattgtttttaaacttaaaaataaggccgggtgtgggggctcacacctgtaatcccagcactttgggaggccgaggtgggtggatcacctgaggtcaggagttcaaaactagcctggccaacatggtgaaaccctgtctctactaaaaatacaaaaattaggccaggcgcagtgggtcatacctgtaatcccagcactttgggaggctgaggagggtggatcacatgaggtaaggagtttgagaccaacctggccaacatggtgaaaccccctcactactaaaaatacaaaaactagccaggcgtggtggcgggtgcctgtaatcccggctactcaggaggctgaggcatgagaatcccttgaacctgggaggcagaggtgcagtgagccgagattgtgccactgcactccagcctgggagatagagtgagactcagtctcaaaaaaaaagaccaaaaattagccaggtgtggtggcaggcgcctgtaatcccagctactcgggaggctgagggaggagaatcacttaaacctgagagacggaggttgcagtgagctgagatcgcaccactgcactccagcctgggtgacagagtaagactcaatctcaaaaaaaaaaaagtcaagtccaaagcccagcctggtccccaacctgcctcatcctcaaccctatccctatctcctttcagccccatcggtggctcaaagacctgaccatgttccctctcccctgaccccggcaggaggctggtggtttggcacctgcagccattccaacctcaacggccagtacttccgctccatcccacagcagcggcagaagcttaagaagggaatcttctggaagacctggcggggccgctactacccgctgcaggccaccaccatgttgatccagcccatggcagcagaggcagcctcctagcgtcctggctgggcctggtcccaggcccacgaaagacggtgactcttggctctgcccgaggatgtggccgttccctgcctgggcaggggctccaaggaggggccatctggaaacttgtggacagagaagaagaccacgactggagaagccccctttctgagtgcaggggggctgcatgcgttgcctcctgagatcgaggctgcaggatatgctcagactctagaggcgtggaccaaggggcatggagcttcactccttgctggccagggagttggggactcagagggaccacttggggccagccagactggcctcaatggcggactcagtcacattgactgacggggaccagggcttgtgtgggtcgagagcgccctcatggtgctggtgctgttgtgtgtaggtcccctggggacacaagcaggcgccaatggtatctgggcggagctcacagagttcttggaataaaagcaacctcagaacactt

SEQ ID NO: 3 - DNA, 17 bp, synthetic construct
  misc_feature 1..17: note = antisense oligonucleotides hybridizing with human ANGPLT4
  source 1..17: mol_type = other DNA
aggctaagttagtggcc

SEQ ID NO: 4 - DNA, 17 bp, synthetic construct
  misc_feature 1..17: note = antisense oligonucleotides hybridizing with human ANGPLT4
  source 1..17: mol_type = other DNA
gccagataggctaagtt

SEQ ID NO: 5 - DNA, 17 bp, synthetic construct
  misc_feature 1..17: note = antisense oligonucleotides hybridizing with human ANGPLT4
  source 1..17: mol_type = other DNA
ctggaaagaatcggatc

SEQ ID NO: 6 - DNA, 17 bp, synthetic construct
  misc_feature 1..17: note = antisense oligonucleotides hybridizing with human ANGPLT4
  source 1..17: mol_type = other DNA
cgctggaaagaatcgga

SEQ ID NO: 7 - DNA, 17 bp, synthetic construct
  misc_feature 1..17: note = antisense oligonucleotides hybridizing with human ANGPLT4
  source 1..17: mol_type = other DNA
gctagtctcgacagcag

SEQ ID NO: 8 - DNA, 17 bp, synthetic construct
  misc_feature 1..17: note = antisense oligonucleotides hybridizing with human ANGPLT4
  source 1..17: mol_type = other DNA
gatcctcatgataggcc

SEQ ID NO: 9 - DNA, 17 bp, synthetic construct
  misc_feature 1..17: note = antisense oligonucleotides hybridizing with human ANGPLT4
  source 1..17: mol_type = other DNA
ggccgtcggagcaccgc

SEQ ID NO: 10 - DNA, 17 bp, synthetic construct
  misc_feature 1..17: note = antisense oligonucleotides hybridizing with human ANGPLT4
  source 1..17: mol_type = other DNA
catgctgtggttcgaga

SEQ ID NO: 11 - DNA, 17 bp, synthetic construct
  misc_feature 1..17: note = antisense oligonucleotides hybridizing with human ANGPLT4
  source 1..17: mol_type = other DNA
cgtgcgccaggacattc

SEQ ID NO: 12 - DNA, 16 bp, synthetic construct
  misc_feature 1..16: note = antisense oligonucleotides hybridizing with human ANGPLT4
  source 1..16: mol_type = other DNA
cgtgcgccaggacatt

SEQ ID NO: 13 - DNA, 17 bp, synthetic construct
  misc_feature 1..17: note = antisense oligonucleotides hybridizing with human ANGPLT4
  source 1..17: mol_type = other DNA
tccgtgcgccaggacat

SEQ ID NO: 14 - DNA, 17 bp, synthetic construct
  misc_feature 1..17: note = antisense oligonucleotides hybridizing with human ANGPLT4
  source 1..17: mol_type = other DNA
ggagtccgtgcgccagg

SEQ ID NO: 15 - DNA, 17 bp, synthetic construct
  misc_feature 1..17: note = antisense oligonucleotides hybridizing with human ANGPLT4
  source 1..17: mol_type = other DNA
tgcgctccgcgtgttcg

SEQ ID NO: 16 - DNA, 16 bp, synthetic construct
  misc_feature 1..16: note = antisense oligonucleotides hybridizing with human ANGPLT4
  source 1..16: mol_type = other DNA
tgcgctccgcgtgttc

SEQ ID NO: 17 - DNA, 16 bp, synthetic construct
  misc_feature 1..16: note = antisense oligonucleotides hybridizing with human ANGPLT4
  source 1..16: mol_type = other DNA
gtgcgctccgcgtgtt

SEQ ID NO: 18 - DNA, 17 bp, synthetic construct
  misc_feature 1..17: note = antisense oligonucleotides hybridizing with human ANGPLT4
  source 1..17: mol_type = other DNA
gtcgaaatgagtctgca

SEQ ID NO: 19 - DNA, 17 bp, synthetic construct
  misc_feature 1..17: note = antisense oligonucleotides hybridizing with human ANGPLT4
  source 1..17: mol_type = other DNA
gcacgtctggaggctca

SEQ ID NO: 20 - DNA, 17 bp, synthetic construct
  misc_feature 1..17: note = antisense oligonucleotides hybridizing with human ANGPLT4
  source 1..17: mol_type = other DNA
ttgagcacgtctggagg

SEQ ID NO: 21 - DNA, 17 bp, synthetic construct
  misc_feature 1..17: note = antisense oligonucleotides hybridizing with human ANGPLT4
  source 1..17: mol_type = other DNA
ggatcgcagtgccgcaa

SEQ ID NO: 22 - DNA, 14 bp, synthetic construct
  misc_feature 1..14: note = non sense artificical sequence
  source 1..14: mol_type = other DNA
aaaaaaaaaaaaaa

SEQ ID NO: 23 - DNA, 17 bp, synthetic construct
  misc_feature 1..17: note = antisense oligonucleotides hybridizing with human ANGPLT4
  source 1..17: mol_type = other DNA
gctgaattcgcaggtgc

SEQ ID NO: 24 - DNA, 16 bp, synthetic construct
  misc_feature 1..16: note = antisense oligonucleotides hybridizing with human ANGPLT4
  source 1..16: mol_type = other DNA
gatcgcagtgccgcaa

SEQ ID NO: 25 - DNA, 17 bp, synthetic construct
  misc_feature 1..17: note = antisense oligonucleotides hybridizing with human ANGPLT4
  source 1..17: mol_type = other DNA
gtgttgtaacctcttgt

SEQ ID NO: 26 - DNA, 17 bp, synthetic construct
  misc_feature 1..17: note = antisense oligonucleotides hybridizing with human ANGPLT4
  source 1..17: mol_type = other DNA
ccgtgttgtaacctctt

SEQ ID NO: 27 - DNA, 17 bp, synthetic construct
  misc_feature 1..17: note = antisense oligonucleotides hybridizing with human ANGPLT4
  source 1..17: mol_type = other DNA
cctcatggtctaggtgc

SEQ ID NO: 28 - DNA, 17 bp, synthetic construct
  misc_feature 1..17: note = antisense oligonucleotides hybridizing with human ANGPLT4
  source 1..17: mol_type = other DNA
cacctcatggtctaggt

SEQ ID NO: 29 - DNA, 17 bp, synthetic construct
  misc_feature 1..17: note = antisense oligonucleotides hybridizing with human ANGPLT4
  source 1..17: mol_type = other DNA
ggcgcctctgaattact

SEQ ID NO: 30 - DNA, 17 bp, synthetic construct
  misc_feature 1..17: note = antisense oligonucleotides hybridizing with human ANGPLT4
  source 1..17: mol_type = other DNA
cgtggcgcctctgaatt

SEQ ID NO: 31 - DNA, 17 bp, synthetic construct
  misc_feature 1..17: note = antisense oligonucleotides hybridizing with human ANGPLT4
  source 1..17: mol_type = other DNA
tcgtggcgcctctgaat

SEQ ID NO: 32 - DNA, 17 bp, synthetic construct
  misc_feature 1..17: note = antisense oligonucleotides hybridizing with human ANGPLT4
  source 1..17: mol_type = other DNA
ccgccttgtaggcttcc

SEQ ID NO: 33 - DNA, 17 bp, synthetic construct
  misc_feature 1..17: note = antisense oligonucleotides hybridizing with human ANGPLT4
  source 1..17: mol_type = other DNA
actcggcgttgccatcc

SEQ ID NO: 34 - DNA, 17 bp, synthetic construct
  misc_feature 1..17: note = antisense oligonucleotides hybridizing with human ANGPLT4
  source 1..17: mol_type = other DNA
gccgtgtcctcgccacc

SEQ ID NO: 35 - DNA, 17 bp, synthetic construct
  misc_feature 1..17: note = antisense oligonucleotides hybridizing with human ANGPLT4
  source 1..17: mol_type = other DNA
gaggtcgtgatcctggt

SEQ ID NO: 36 - DNA, 17 bp, synthetic construct
  misc_feature 1..17: note = antisense oligonucleotides hybridizing with human ANGPLT4
  source 1..17: mol_type = other DNA
gcggaggtcgtgatcct

SEQ ID NO: 37 - DNA, 17 bp, synthetic construct
  misc_feature 1..17: note = antisense oligonucleotides hybridizing with human ANGPLT4
  source 1..17: mol_type = other DNA
cctgcggaggtcgtgat

SEQ ID NO: 38 - DNA, 17 bp, synthetic construct
  misc_feature 1..17: note = antisense oligonucleotides hybridizing with human ANGPLT4
  source 1..17: mol_type = other DNA
ctcttggcgcagttctt

SEQ ID NO: 39 - DNA, 17 bp, synthetic construct
  misc_feature 1..17: note = antisense oligonucleotides hybridizing with human ANGPLT4
  source 1..17: mol_type = other DNA
gctcttggcgcagttct

SEQ ID NO: 40 - DNA, 17 bp, synthetic construct
  misc_feature 1..17: note = antisense oligonucleotides hybridizing with human ANGPLT4
  source 1..17: mol_type = other DNA
ggctcttggcgcagttc

SEQ ID NO: 41 - DNA, 17 bp, synthetic construct
  misc_feature 1..17: note = antisense oligonucleotides hybridizing with human ANGPLT4
  source 1..17: mol_type = other DNA
ggtgccaaaccaccagc

SEQ ID NO: 42 - DNA, 17 bp, synthetic construct
  misc_feature 1..17: note = antisense oligonucleotides hybridizing with human ANGPLT4
  source 1..17: mol_type = other DNA
ggagcggaagtactggc

SEQ ID NO: 43 - DNA, 17 bp, synthetic construct
  misc_feature 1..17: note = antisense oligonucleotides hybridizing with human ANGPLT4
  source 1..17: mol_type = other DNA
atggagcggaagtactg

SEQ ID NO: 44 - DNA, 17 bp, synthetic construct
  misc_feature 1..17: note = antisense oligonucleotides hybridizing with human ANGPLT4
  source 1..17: mol_type = other DNA
ggatggagcggaagtac

SEQ ID NO: 45 - DNA, 17 bp, synthetic construct
  misc_feature 1..17: note = antisense oligonucleotides hybridizing with human ANGPLT4
  source 1..17: mol_type = other DNA
ggctggatcaacatggt

SEQ ID NO: 46 - DNA, 17 bp, synthetic construct
  misc_feature 1..17: note = antisense oligonucleotides hybridizing with human ANGPLT4
  source 1..17: mol_type = other DNA
atgtgactgagtccgcc

SEQ ID NO: 47 - DNA, 17 bp, synthetic construct
  misc_feature 1..17: note = antisense oligonucleotides hybridizing with human ANGPLT4
  source 1..17: mol_type = other DNA
caatgtgactgagtccg

SEQ ID NO: 48 - DNA, 17 bp, synthetic construct
  misc_feature 1..17: note = antisense oligonucleotides hybridizing with human ANGPLT4
  source 1..17: mol_type = other DNA
gaactctgtgagctccg

SEQ ID NO: 49 - DNA, 17 bp, synthetic construct
  misc_feature 1..17: note = antisense oligonucleotides hybridizing with human ANGPLT4
  source 1..17: mol_type = other DNA
ctggtggactaacacac

SEQ ID NO: 50 - DNA, 17 bp, synthetic construct
  misc_feature 1..17: note = antisense oligonucleotides hybridizing with human ANGPLT4
  source 1..17: mol_type = other DNA
tggacctgacaaggaga

SEQ ID NO: 51 - DNA, 16 bp, synthetic construct
  misc_feature 1..16: note = antisense oligonucleotides hybridizing with human ANGPLT4
  source 1..16: mol_type = other DNA
cacacggcatgtaagg

SEQ ID NO: 52 - DNA, 17 bp, synthetic construct
  misc_feature 1..17: note = antisense oligonucleotides hybridizing with human ANGPLT4
  source 1..17: mol_type = other DNA
aggctagtctcgacagc

SEQ ID NO: 53 - DNA, 17 bp, synthetic construct
  misc_feature 1..17: note = antisense oligonucleotides hybridizing with human ANGPLT4
  source 1..17: mol_type = other DNA
gatcgcagtgccgcaat

SEQ ID NO: 54 - DNA, 17 bp, synthetic construct
  misc_feature 1..17: note = antisense oligonucleotides hybridizing with human ANGPLT4
  source 1..17: mol_type = other DNA
cgtgttgtaacctcttg

SEQ ID NO: 55 - DNA, 15 bp, synthetic construct
  misc_feature 1..15: note = antisense oligonucleotides hybridizing with human ANGPLT4
  source 1..15: mol_type = other DNA
gatcgcagtgccgca

SEQ ID NO: 56 - DNA, 15 bp, synthetic construct
  misc_feature 1..15: note = antisense oligonucleotides hybridizing with human ANGPLT4
  source 1..15: mol_type = other DNA
ggatcgcagtgccgc

SEQ ID NO: 57 - DNA, 18 bp, synthetic construct
  misc_feature 1..18: note = oligonucleotide negative control
  modified_base 1..17: mod_base = OTHER; note = nucleotide may be modified with phosphorothioate (PTO)
  modified_base 1..3: mod_base = OTHER; note = nucleotide may be modified as locked nucleic acid (LNA)
  modified_base 15..17: mod_base = OTHER; note = nucleotide may be modified as locked nucleic acid (LNA)
  source 1..18: mol_type = other DNA
cgtttaggctatgtactt

SEQ ID NO: 58 - DNA, 1916 bp, Mus musculus
  source 1..1916: mol_type = genomic DNA
gctttataaagtggggctttaggtgcaaccgtgaaacgcttatgagctacgggctccagatcttcttctgcaccagagcaagtctaagtctgagccggctcccccagaactccagctgctgggtcttgaactcctgcgttccggagtcctagcgttgctgcacccaaggccacccccagaatcatgcgctgcgctccgacagcaggcgctgccctggtgctatgcgcggctactgcggggcttttgagcgcgcaagggcgccctgcacagccagagccaccgcgctttgcatcctgggacgagatgaacttgctggctcacgggctgctacagctcggccatgggctgcgcgaacacgtggagcgcacccgtgggcagctgggcgcgctggagcgccgcatggctgcctgtggtaacgcttgtcaggggcccaagggaaaagatgcacccttcaaagactccgaggatagagtccctgaaggccagactcctgagactctgcagagtttgcagactcagctcaaggctcaaaacagcaagatccagcaattgttccagaaggtggcccagcagcagagatacctatcaaagcagaatctgagaatacagaatcttcagagccagatagacctcttggcccccacgcacctagacaatggagtagacaagacttcgaggggaaagaggcttcccaagatgacccagctcattggcttgactcccaacgccacccacttacacaggccgccccgggactgccaggaactcttccaagaaggggagcggcacagtggacttttccagatccagcctctggggtctccaccatttttggtcaactgtgagatgacttcagatggaggctggacagtgattcagagacgcctgaacggctctgtggacttcaaccagtcctgggaagcctacaaggatggcttcggagatccccaaggcgagttctggctgggcctggaaaagatgcacagcatcacagggaaccgaggaagccaattggctgtgcagctccaggactgggatggcaatgccaaattgctccaatttcccatccatttggggggtgaggacacagcctacagcctgcagctcactgagcccacggccaatgagctgggtgccaccaatgtttcccccaatggcctttccctgcccttctctacttgggaccaagaccatgacctccgtggggaccttaactgtgccaagagcctctctggtggctggtggtttggtacctgtagccattccaatctcaatggacaatacttccactctatcccacggcaacggcaggagcgtaaaaagggtatcttctggaaaacatggaagggccgctactatcctctgcaggctaccaccctgctgatccagcccatggaggctacagcagcctcttagcctcctcactggagcctggttccaggcctaagaagacagtgactttggttgtggccctgagatttggccattctctgctgggggcaggagctctaagtagggctatctgcgtcttgtggacaaagaagaagcccgtaactggagagactggaggaccccttttccgtgttggggtctgcaagcattgttgtctgaaacagtcagagcaacaggaaacaaatggcccagatccagaaaacatgggctcgaggggcactgaatatcacttctcgcctaccagagaagttggggatgcagagggaccactacagtccaactagctgggcccttaatggcggactcagtcatattgactgactggagacagggtgccaggagccctggatacactcatggtgctgttgtaggtgctgtggatgcacaggtgctaactgtggttcccaggcacagctcacagcattcttacaataaaaacaacctcagaacaaaaaaaaaaaaaa

SEQ ID NO: 59 - DNA, 7826 bp, Mus musculus
  source 1..7826: mol_type = genomic DNA
gctttataaagtggggctttaggtgcaaccgtgaaacgcttatgagctacgggctccagatcttcttctgcaccagagcaagtctaagtctgagccggctcccccagaactccagctgctgggtcttgaactcctgcgttccggagtcctagcgttgctgcacccaaggccacccccagaatcatgcgctgcgctccgacagcaggcgctgccctggtgctatgcgcggctactgcggggcttttgagcgcgcaagggcgccctgcacagccagagccaccgcgctttgcatcctgggacgagatgaacttgctggctcacgggctgctacagctcggccatgggctgcgcgaacacgtggagcgcacccgtgggcagctgggcgcgctggagcgccgcatggctgcctgtggtaacgcttgtcaggggcccaagggaaaagatgcacccttcaaagactccgaggatagagtccctgaaggccagactcctgagactctgcagagtttgcaggtaggcgcatctactaggactctgactctacttagactaacgagtctagtactccaggacctgggtggagaagggcctcagagcagactgtgaaagggtagaagggagggtgaataagaggaggttgccgacataaagccaggtcttcactagccttgcatatcttcagactcagctcaaggctcaaaacagcaagatccagcaattgttccagaaggtggcccagcagcagagatacctatcaaagcagaatctgagaatacagaatcttcagagccaggtaattaccccagcaattggcccaaatgggaaagaggaaacaaagtgggggtgaaatgtagtgatgaaatgtggctaagcagttgttatggcatgagtcaaaagatctaaccacccgtttcctgcccggtcttagatagacctcttggcccccacgcacctagacaatggagtagacaagacttcgaggggaaagaggcttcccaagatgacccagctcattggcttgactcccaacgccacccacttacacagtgagtatctctggtctttgctgtcatctggcaactccccaaccaccccacttgccattccaatccttagccttcttgtcaggtccaccttaataggaaagaaagagattctggccttgggttcctgtgggctcactaggctctcatcaagggtatttttatatattgcaccctcttcacttatgatcctgcttggccagaccaccccaccattctttcccagcaagaatcttcccaaaatcttattagccgttaaccagaacaagtagaggaaggcagatcataaggagctaaagtttcaggggttctgggagatggtggtgtagctcagggacatcatgcaaaggaatccagggctgtgtgtggatgtgtgtgcgttcccgaggtttggaaccctccaacatctcttgatgtaactataaaagggaaaaccagagtaagcacacccccaccccggctcctagactagacacatcctcttacatcttacagatacagatcctttgtcctgtatgcttccatccagtcacatacacatatatacataacagtttcgatcacaatttctaggtcttagattgtggatgtccatgcccaatactttgtttcaaattgaagtgtgtgtggagctacgcagtgcgggatgggcgggtgggggatggggggcacagagtcagaggctcccagttccaaccctgagttcatgcctattcgttcacccttcttgacatctgtggctctccacagccaactaggtgaaagtttggatatccccttcacaccctaaggctgcttgctggctttcagcccaatcctccttagacttaattcctcccctggcttttacttaggcaagtacctaggcatggcgagggtcatggatgagcttttccagggtcggcaggcataggttctggatgggtgatgtggtggaagagaagagctgagggggtggttttgtggctttggaactcccagactcagcctagccaagtagaggaaagttcagagctggagagacaaacagctggccctaatgggaaccacatgggtggtttggcagtgtgcctgtcccgattggatgagaggaaagtaggggaaagggagctagctgcccgagggattggaaagtatacttcccatctttctgggtctgcccccactcctggcagtgcagacggagctggctggcagaaagtgcctgcatgcccctcccccagtgacctttctcctactttccctggctgggctgggggtggttcttcctgaatttagaggacttgtcaaggccaagttctttctctcctcctctcctctttttcttttcttcctcttcccccttcttctggtaacagacatagccgtatcccacacacacacccagcctcagtctcccagtcccactgtcagcatcttctactaattcagagtacccctttgctcagtcagctcagctcttgccttaccccagatccaccccgtccattgtttgaagtcttcactgaaacactgactgtggggtaggctttaggtggttacaggtccctactgtggacaaacttcctcctcgtctctggcctcagtgggaggagtggggacatgcctccagatgactcttcatcagcgacaatacctctgttcacttttgggagtctaacagggcttgagagagtggaatagcatccttttagaagctgagacccagagaaaggaatgggaaaatggaatccctggcatcaggaccatgtgctgattgtcaataacaggaaggtgtgatacatgggaaaaaggctcagggagagaagcctttgtgacctgagagggtagacaagcagagtgggaagagtgaagattggtcaagggactgaccgttccttagtgtgccttgaggaccctactggagaatgctataatgaggcaggaacgagtttaggcaaatcaccctggggctcatcctctaccacccagccttcacactcaccagtctcctgaaatcactgggggcttctctcctgcttcactctctccctttgtctactttcagggccgccccgggactgccaggaactcttccaagaaggggagcggcacagtggacttttccagatccagcctctggggtctccaccatttttggtcaactgtgagatgacttcaggtaggatgtgctgacacccacccccccaaggagcctccttgccatgcacagccctgatgtcataaaataaagccatgtatagatcaataattacaagcacttacctagcttgtataagctcctgagatccttccacagtaacacacaccctattatgcagcttgtaggatgtagcctgtaggaggtatatagataatcttcttccctattgacaggcatcgcaagctcagtgataggtttctgtggttaaggtgtacagctgtccaggcctagtcatctacaaggtgagatcaaggccagcctgggtaacttagtataaccctgtcatgcaataacaaaatataagtgagctgggggcatagcttaatgggaaagtgcctcctacaatgtacaagaccctaaattcaatgcatagaaccacagttggatatggtgacttgtgcctatatttataatcccaatacttgggaggttgaggcaaaatgattgttgaaagtgcaaggccagccttatctcagtcttcatgggctgggaataaagctcagttggtaaagcgcttccattgaatgtatgaagccctggcttccatctccaacactgcataaaatgggtatgatagtgcaagtctgctacccaaaactctggaggtggtagcaggctgatgaggagtttgagatcatccacagttacatagtgagttgaaggacagcttgggctataggaaaaaggtagtctaaggtagagactctgtttcaaacaacaaaacacatatactcctggttcctgcaggctcctaggatagaagtctgttctgatcccaccccctgcggggactgatgagtgtgttgcccttcctgggattgtatgggagcatgatattaggcttgcaagctaggtagggctatcagtttccctgtgagaagggacttctggtgactttttgtctttctgggcagatggaggctggacagtgattcagagacgcctgaacggctctgtggacttcaaccagtcctgggaagcctacaaggatggcttcggagatccccaaggtaggtgtttctctggaggccatagtcatggaaggagcaaagggtgcgagagttgagcctggctcacatatgatttctcttgattcaggcgagttctggctgggcctggaaaagatgcacagcatcacagggaaccgaggaagccaattggctgtgcagctccaggactgggatggcaatgccaaattgctccaatttcccatccatttggggggtgaggacacagcctacagcctgcagctcactgagcccacggccaatgagctgggtgccaccaatgtttcccccaatggcctttccctgcccttctctacttgggaccaagaccatgacctccgtggggaccttaactgtgccaagagcctctctggtaagcaggttttattcccactgtagcctacattcagtcccaaagtgtgtatccatgccctgccccccttttctccttgcctcctgtgtgcctatgggccagtcattgaattaatctctgctgttttcagtttccctgtctttaagtgaacataatcatggtgcctgcttttgaaaattcaactgagaacatttgtgggtgtgtagctgccacagggcaaagccaagacaaacccttgtcttattcttttcaattctgaggtatagggtcttgtgccattctggcacagagctacaccctgacccctggtgttttgtttttgttgtctgtttgactcagggtcttatatagctctagctggccttgaacttgttatacagctaaagataagcttaaagggtcagcctcggagctggaaagatggctcagtggttaagagcactgactgctcttcccaggggtcctgagttcaattcccagcaactccatggtggctcacaaccacctccaatggggtctgatgccctcttctggtgtgtctgaagagagcaatggtgtattcatatacattaaataaataaaccatttaaaaagggaggggggcatcagcctctaactcctgagtgttggggtaacaggcatgtgccattgtgctcctgaggatcaatcccacaattccatgtctggtaggcaagcactgtaacaaatgagctacagtactagctctttttctgcttcacttattcagtcaggatcaaattataaagagcaggctggcctcaaacttcctatcatactgctgagcactgtgactacaaatttctacccacaaactgcttcatagtgtagctcatttggcagagaacctacctaacatgagtgaaggcctaggtttcattacccataccatataaaacacacatggttgtgcaatgtcaaccatagactcagaaagaggaggcaggtaaagcagacattttaaattgtctttggccacgtggagagtttgaggccagcccgataggagaccccgtcacaaaacaaaaataggacttatgagatggctcagccagtaacagtgtttgcctacaatcctgaagacctaagtttgatctccaagactcacatagtagaaagagatcactggctcgctcccacaagctgtcctctgaccttcatacccactgtggcatgtacacccacacacatatacacgggaacacaaagtaaataaatgtaataaattctaaaggtgtaaaatccaaagttcatcttgtctccaactgtgctctctctctctctctctcctctctctctctctctctctctcagtatggaaacccaagaccttgaccacatctcctgttctttaaccctataggtggctggtggtttggtacctgtagccattccaatctcaatggacaatacttccactctatcccacggcaacggcaggagcgtaaaaagggtatcttctggaaaacatggaagggccgctactatcctctgcaggctaccaccctgctgatccagcccatggaggctacagcagcctcttagcctcctcactggagcctggttccaggcctaagaagacagtgactttggttgtggccctgagatttggccattctctgctgggggcaggagctctaagtagggctatctgcgtcttgtggacaaagaagaagcccgtaactggagagactggaggaccccttttccgtgttggggtctgcaagcattgttgtctgaaacagtcagagcaacaggaaacaaatggcccagatccagaaaacatgggctcgaggggcactgaatatcacttctcgcctaccagagaagttggggatgcagagggaccactacagtccaactagctgggcccttaatggcggactcagtcatattgactgactggagacagggtgccaggagccctggatacactcatggtgctgttgtaggtgctgtggatgcacaggtgctaactgtggttcccaggcacagctcacagcattcttacaataaaaacaacctcagaacattttgttctctgttgtttcatttgatttttcaaagtgaatagtttcaaagttcaagtaaacatgttcctcggacatcgtattcccagatccgttaaggacagaactggttggctattccttcccagtgatttcagcttccttcttttagtatttcatgatgtgagcctctcttgtttatatttcaaaatctcaaaacaggtccagggagatggctcagtgattaggaacattcgttcttccagagggcctgggtttggttcccagcctttacatagcagctaacaatagcctataactctacttcaagggggtccaatgccgcctctgacctctactggctcctgtacaaatgtgataatatgcaaatatttaggcactcatatagaaaagaaagtattgtttaaaaaacagagttagggaaatggcttaatgattccaaacacttgctgtctaagcctggtgactgagttcaagcacccaaaaggtcaaaggacagaacagattccgcaaagttggcctttgaccaccacatacaagccatggcacttgggctgtcacacagatatatacacaataattgttttttttttaatttttaaaagttaaaaatcatataactcatgcagtccaatcattagggaagttggtgatagagacaagtaaaaagtctttctgatcagtactcggtggggtacacacagatctccagcccctgggagctggacataggagctttgcaaactctaagccagactaggcaatacaacaagatcctgtatcacaaacagggtgagtactgtagatgtagctcaactggacatacgaagcatgcacagaccctgggttctttcccagcagcactgcataaataaagtatagcgctagataacactgtaatgctcgtatttgggaggtggaggcatgaggattagaagttgaggtaacctgggctacaagaaagaaaaagaagagagaaaagcaaaatgagatgaagttaattttagaaatctaaacccgatgtcatattccatacttgtaatttcagcacttggggagctgaggcagggggaccagaattaccatgagtttgagtccaacttaggctatatagtaagaccttgactaataaaaacaaagacgttaaaaaag

SEQ ID NO: 60 - DNA, 15 bp, synthetic construct
  misc_feature 1..15: note = antisense oligonucleotides hybridizing with murine ANGPLT4
  source 1..15: mol_type = other DNA
gttgcacctaaagcc

SEQ ID NO: 61 - DNA, 17 bp, synthetic construct
  misc_feature 1..17: note = antisense oligonucleotides hybridizing with murine ANGPLT4
  source 1..17: mol_type = other DNA
acggttgcacctaaagc

SEQ ID NO: 62 - DNA, 16 bp, synthetic construct
  misc_feature 1..16: note = antisense oligonucleotides hybridizing with murine ANGPLT4
  source 1..16: mol_type = other DNA
acggttgcacctaaag

SEQ ID NO: 63 - DNA, 16 bp, synthetic construct
  misc_feature 1..16: note = antisense oligonucleotides hybridizing with murine ANGPLT4
  source 1..16: mol_type = other DNA
tcacggttgcacctaa

SEQ ID NO: 64 - DNA, 16 bp, synthetic construct
  misc_feature 1..16: note = antisense oligonucleotides hybridizing with murine ANGPLT4
  source 1..16: mol_type = other DNA
ttcacggttgcaccta

SEQ ID NO: 65 - DNA, 17 bp, synthetic construct
  misc_feature 1..17: note = antisense oligonucleotides hybridizing with murine ANGPLT4
  source 1..17: mol_type = other DNA
ataagcgtttcacggtt

SEQ ID NO: 66 - DNA, 17 bp, synthetic construct
  misc_feature 1..17: note = antisense oligonucleotides hybridizing with murine ANGPLT4
  source 1..17: mol_type = other DNA
cataagcgtttcacggt

SEQ ID NO: 67 - DNA, 17 bp, synthetic construct
  misc_feature 1..17: note = antisense oligonucleotides hybridizing with murine ANGPLT4
  source 1..17: mol_type = other DNA
cgtagctcataagcgtt

SEQ ID NO: 68 - DNA, 16 bp, synthetic construct
  misc_feature 1..16: note = antisense oligonucleotides hybridizing with murine ANGPLT4
  source 1..16: mol_type = other DNA
gctaggactccggaac

SEQ ID NO: 69 - DNA, 17 bp, synthetic construct
  misc_feature 1..17: note = antisense oligonucleotides hybridizing with murine ANGPLT4
  source 1..17: mol_type = other DNA
acgctaggactccggaa

SEQ ID NO: 70 - DNA, 15 bp, synthetic construct
  misc_feature 1..15: note = antisense oligonucleotides hybridizing with murine ANGPLT4
  source 1..15: mol_type = other DNA
aacgctaggactccg

SEQ ID NO: 71 - DNA, 15 bp, synthetic construct
  misc_feature 1..15: note = antisense oligonucleotides hybridizing with murine ANGPLT4
  source 1..15: mol_type = other DNA
agcgcatgattctgg

SEQ ID NO: 72 - DNA, 17 bp, synthetic construct
  misc_feature 1..17: note = antisense oligonucleotides hybridizing with murine ANGPLT4
  source 1..17: mol_type = other DNA
cggagcgcagcgcatga

SEQ ID NO: 73 - DNA, 17 bp, synthetic construct
  misc_feature 1..17: note = antisense oligonucleotides hybridizing with murine ANGPLT4
  source 1..17: mol_type = other DNA
agccgcgcatagcacca

SEQ ID NO: 74 - DNA, 16 bp, synthetic construct
  misc_feature 1..16: note = antisense oligonucleotides hybridizing with murine ANGPLT4
  source 1..16: mol_type = other DNA
tagccgcgcatagcac

SEQ ID NO: 75 - DNA, 17 bp, synthetic construct
  misc_feature 1..17: note = antisense oligonucleotides hybridizing with murine ANGPLT4
  source 1..17: mol_type = other DNA
agtagccgcgcatagca

SEQ ID NO: 76 - DNA, 17 bp, synthetic construct
  misc_feature 1..17: note = antisense oligonucleotides hybridizing with murine ANGPLT4
  source 1..17: mol_type = other DNA
cagtagccgcgcatagc

SEQ ID NO: 77 - DNA, 16 bp, synthetic construct
  misc_feature 1..16: note = antisense oligonucleotides hybridizing with murine ANGPLT4
  source 1..16: mol_type = other DNA
cagtagccgcgcatag

SEQ ID NO: 78 - DNA, 16 bp, synthetic construct
  misc_feature 1..16: note = antisense oligonucleotides hybridizing with murine ANGPLT4
  source 1..16: mol_type = other DNA
gcagtagccgcgcata

SEQ ID NO: 79 - DNA, 15 bp, synthetic construct
  misc_feature 1..15: note = antisense oligonucleotides hybridizing with murine ANGPLT4
  source 1..15: mol_type = other DNA
ccttgcgcgctcaaa

SEQ ID NO: 80 - DNA, 16 bp, synthetic construct
  misc_feature 1..16: note = antisense oligonucleotides hybridizing with murine ANGPLT4
  source 1..16: mol_type = other DNA
gatgcaaagcgcggtg

SEQ ID NO: 81 - DNA, 17 bp, synthetic construct
  misc_feature 1..17: note = antisense oligonucleotides hybridizing with murine ANGPLT4
  source 1..17: mol_type = other DNA
aggatgcaaagcgcggt

SEQ ID NO: 82 - DNA, 16 bp, synthetic construct
  misc_feature 1..16: note = antisense oligonucleotides hybridizing with murine ANGPLT4
  source 1..16: mol_type = other DNA
ccacgtgttcgcgcag

SEQ ID NO: 83 - DNA, 17 bp, synthetic construct
  misc_feature 1..17: note = antisense oligonucleotides hybridizing with murine ANGPLT4
  source 1..17: mol_type = other DNA
ctccacgtgttcgcgca

SEQ ID NO: 84 - DNA, 17 bp, synthetic construct
  misc_feature 1..17: note = antisense oligonucleotides hybridizing with murine ANGPLT4
  source 1..17: mol_type = other DNA
tgcgctccacgtgttcg

SEQ ID NO: 85 - DNA, 16 bp, synthetic construct
  misc_feature 1..16: note = antisense oligonucleotides hybridizing with murine ANGPLT4
  source 1..16: mol_type = other DNA
tgcgctccacgtgttc

SEQ ID NO: 86 - DNA, 15 bp, synthetic construct
  misc_feature 1..15: note = antisense oligonucleotides hybridizing with murine ANGPLT4
  source 1..15: mol_type = other DNA
tgcgctccacgtgtt

SEQ ID NO: 87 - DNA, 16 bp, synthetic construct
  misc_feature 1..16: note = antisense oligonucleotides hybridizing with murine ANGPLT4
  source 1..16: mol_type = other DNA
atgcggcgctccagcg

SEQ ID NO: 88 - DNA, 17 bp, synthetic construct
  misc_feature 1..17: note = antisense oligonucleotides hybridizing with murine ANGPLT4
  source 1..17: mol_type = other DNA
ctgacaagcgttaccac

SEQ ID NO: 89 - DNA, 17 bp, synthetic construct
  misc_feature 1..17: note = antisense oligonucleotides hybridizing with murine ANGPLT4
  source 1..17: mol_type = other DNA
cctgacaagcgttacca

SEQ ID NO: 90 - DNA, 15 bp, synthetic construct
  misc_feature 1..15: note = antisense oligonucleotides hybridizing with murine ANGPLT4
  source 1..15: mol_type = other DNA
cctgacaagcgttac

SEQ ID NO: 91 - DNA, 16 bp, synthetic construct
  misc_feature 1..16: note = antisense oligonucleotides hybridizing with murine ANGPLT4
  source 1..16: mol_type = other DNA
attgtctaggtgcgtg

SEQ ID NO: 92 - DNA, 17 bp, synthetic construct
  misc_feature 1..17: note = antisense oligonucleotides hybridizing with murine ANGPLT4
  source 1..17: mol_type = other DNA
ccattgtctaggtgcgt

SEQ ID NO: 93 - DNA, 17 bp, synthetic construct
  misc_feature 1..17: note = antisense oligonucleotides hybridizing with murine ANGPLT4
  source 1..17: mol_type = other DNA
cgttcaggcgtctctga

SEQ ID NO: 94 - DNA, 16 bp, synthetic construct
  misc_feature 1..16: note = antisense oligonucleotides hybridizing with murine ANGPLT4
  source 1..16: mol_type = other DNA
agagccgttcaggcgt

SEQ ID NO: 95 - DNA, 15 bp, synthetic construct
  misc_feature 1..15: note = antisense oligonucleotides hybridizing with murine ANGPLT4
  source 1..15: mol_type = other DNA
gctcattggccgtgg

SEQ ID NO: 96 - DNA, 17 bp, synthetic construct
  misc_feature 1..17: note = antisense oligonucleotides hybridizing with murine ANGPLT4
  source 1..17: mol_type = other DNA
agtggaagtattgtcca

SEQ ID NO: 97 - DNA, 17 bp, synthetic construct
  misc_feature 1..17: note = antisense oligonucleotides hybridizing with murine ANGPLT4
  source 1..17: mol_type = other DNA
tacgctcctgccgttgc

SEQ ID NO: 98 - DNA, 17 bp, synthetic construct
  misc_feature 1..17: note = antisense oligonucleotides hybridizing with murine ANGPLT4
  source 1..17: mol_type = other DNA
ttacgctcctgccgttg

SEQ ID NO: 99 - DNA, 17 bp, synthetic construct
  misc_feature 1..17: note = antisense oligonucleotides hybridizing with murine ANGPLT4
  source 1..17: mol_type = other DNA
tttttacgctcctgccg

SEQ ID NO: 100 - DNA, 15 bp, synthetic construct
  misc_feature 1..15: note = antisense oligonucleotides hybridizing with murine ANGPLT4
  source 1..15: mol_type = other DNA
ttttacgctcctgcc

SEQ ID NO: 101 - DNA, 17 bp, synthetic construct
  misc_feature 1..17: note = antisense oligonucleotides hybridizing with murine ANGPLT4
  source 1..17: mol_type = other DNA
agaggatagtagcggcc

SEQ ID NO: 102 - DNA, 17 bp, synthetic construct
  misc_feature 1..17: note = antisense oligonucleotides hybridizing with murine ANGPLT4
  source 1..17: mol_type = other DNA
acaagacgcagatagcc

SEQ ID NO: 103 - DNA, 17 bp, synthetic construct
  misc_feature 1..17: note = antisense oligonucleotides hybridizing with murine ANGPLT4
  source 1..17: mol_type = other DNA
ggcgagaagtgatattc

SEQ ID NO: 104 - DNA, 17 bp, synthetic construct
  misc_feature 1..17: note = antisense oligonucleotides hybridizing with murine ANGPLT4
  source 1..17: mol_type = other DNA
taggcgagaagtgatat

SEQ ID NO: 105 - DNA, 16 bp, synthetic construct
  misc_feature 1..16: note = antisense oligonucleotides hybridizing with murine ANGPLT4
  source 1..16: mol_type = other DNA
gtaggcgagaagtgat

SEQ ID NO: 106 - DNA, 16 bp, synthetic construct
  misc_feature 1..16: note = antisense oligonucleotides hybridizing with murine ANGPLT4
  source 1..16: mol_type = other DNA
gagtccgccattaagg

SEQ ID NO: 107 - DNA, 17 bp, synthetic construct
  misc_feature 1..17: note = antisense oligonucleotides hybridizing with murine ANGPLT4
  source 1..17: mol_type = other DNA
actgagtccgccattaa

SEQ ID NO: 108 - DNA, 17 bp, synthetic construct
  misc_feature 1..17: note = antisense oligonucleotides hybridizing with murine ANGPLT4
  source 1..17: mol_type = other DNA
atatgactgagtccgcc

SEQ ID NO: 109 - DNA, 17 bp, synthetic construct
  misc_feature 1..17: note = antisense oligonucleotides hybridizing with murine ANGPLT4
  source 1..17: mol_type = other DNA
aatatgactgagtccgc

SEQ ID NO: 110 - DNA, 16 bp, synthetic construct
  misc_feature 1..16: note = antisense oligonucleotides hybridizing with murine ANGPLT4
  source 1..16: mol_type = other DNA
cgctaggactccggaa

SEQ ID NO: 111 - DNA, 17 bp, synthetic construct
  misc_feature 1..17: note = antisense oligonucleotides hybridizing with murine ANGPLT4
  source 1..17: mol_type = other DNA
aacgctaggactccgga

SEQ ID NO: 112 - DNA, 16 bp, synthetic construct
  misc_feature 1..16: note = antisense oligonucleotides hybridizing with murine ANGPLT4
  source 1..16: mol_type = other DNA
aacgctaggactccgg

SEQ ID NO: 113 - DNA, 16 bp, synthetic construct
  misc_feature 1..16: note = antisense oligonucleotides hybridizing with murine ANGPLT4
  source 1..16: mol_type = other DNA
caacgctaggactccg

SEQ ID NO: 114 - DNA, 17 bp, synthetic construct
  misc_feature 1..17: note = antisense oligonucleotides hybridizing with murine ANGPLT4
  source 1..17: mol_type = other DNA
gcaacgctaggactccg

SEQ ID NO: 115 - DNA, 15 bp, synthetic construct
  misc_feature 1..15: note = antisense oligonucleotides hybridizing with murine ANGPLT4
  source 1..15: mol_type = other DNA
gtagccgcgcatagc

SEQ ID NO: 116 - DNA, 16 bp, synthetic construct
  misc_feature 1..16: note = antisense oligonucleotides hybridizing with murine ANGPLT4
  source 1..16: mol_type = other DNA
agtagccgcgcatagc

SEQ ID NO: 117 - DNA, 15 bp, synthetic construct
  misc_feature 1..15: note = antisense oligonucleotides hybridizing with murine ANGPLT4
  source 1..15: mol_type = other DNA
agtagccgcgcatag

SEQ ID NO: 118 - DNA, 17 bp, synthetic construct
  misc_feature 1..17: note = antisense oligonucleotides hybridizing with murine ANGPLT4
  source 1..17: mol_type = other DNA
gcagtagccgcgcatag

SEQ ID NO: 119 - DNA, 15 bp, synthetic construct
  misc_feature 1..15: note = antisense oligonucleotides hybridizing with murine ANGPLT4
  source 1..15: mol_type = other DNA
cagtagccgcgcata

SEQ ID NO: 120 - DNA, 17 bp, synthetic construct
  misc_feature 1..17: note = antisense oligonucleotides hybridizing with murine ANGPLT4
  source 1..17: mol_type = other DNA
ccgcagtagccgcgcat

SEQ ID NO: 121 - DNA, 16 bp, synthetic construct
  misc_feature 1..16: note = antisense oligonucleotides hybridizing with murine ANGPLT4
  source 1..16: mol_type = other DNA
ccttgcgcgctcaaaa

SEQ ID NO: 122 - DNA, 16 bp, synthetic construct
  misc_feature 1..16: note = antisense oligonucleotides hybridizing with murine ANGPLT4
  source 1..16: mol_type = other DNA
ccttgcgcgctcaaaa

SEQ ID NO: 123 - DNA, 16 bp, synthetic construct
  misc_feature 1..16: note = antisense oligonucleotides hybridizing with murine ANGPLT4
  source 1..16: mol_type = other DNA
atgcaaagcgcggtgg

SEQ ID NO: 124 - DNA, 15 bp, synthetic construct
  misc_feature 1..15: note = antisense oligonucleotides hybridizing with murine ANGPLT4
  source 1..15: mol_type = other DNA
atgcaaagcgcggtg

SEQ ID NO: 125 - DNA, 15 bp, synthetic construct
  misc_feature 1..15: note = antisense oligonucleotides hybridizing with murine ANGPLT4
  source 1..15: mol_type = other DNA
cgctccacgtgttcg

SEQ ID NO: 126 - DNA, 16 bp, synthetic construct
  misc_feature 1..16: note = antisense oligonucleotides hybridizing with murine ANGPLT4
  source 1..16: mol_type = other DNA
gcgctccacgtgttcg

SEQ ID NO: 127 - DNA, 17 bp, synthetic construct
  misc_feature 1..17: note = antisense oligonucleotides hybridizing with murine ANGPLT4
  source 1..17: mol_type = other DNA
tgagtccgccattaagg

SEQ ID NO: 128 - DNA, 16 bp, synthetic construct
  misc_feature 1..16: note = antisense oligonucleotides hybridizing with murine ANGPLT4
  source 1..16: mol_type = other DNA
atgactgagtccgcca

SEQ ID NO: 129 - DNA, 16 bp, synthetic construct
  misc_feature 1..16: note = antisense oligonucleotides hybridizing with murine ANGPLT4
  source 1..16: mol_type = other DNA
tatgactgagtccgcc

SEQ ID NO: 130 - DNA, 17 bp, synthetic construct
  misc_feature 1..17: note = antisense oligonucleotides hybridizing with murine ANGPLT4
  source 1..17: mol_type = other DNA
aatatgactgagtccgc

SEQ ID NO: 131 - DNA, 16 bp, synthetic construct
  misc_feature 1..16: note = antisense oligonucleotides hybridizing with murine ANGPLT4
  source 1..16: mol_type = other DNA
aatatgactgagtccg

SEQ ID NO: 132 - DNA, 17 bp, synthetic construct
  misc_feature 1..17: note = antisense oligonucleotides hybridizing with murine ANGPLT4
  source 1..17: mol_type = other DNA
cctagtagatgcgccta

SEQ ID NO: 133 - DNA, 17 bp, synthetic construct
  misc_feature 1..17: note = antisense oligonucleotides hybridizing with murine ANGPLT4
  source 1..17: mol_type = other DNA
tcgttagtctaagtaga

SEQ ID NO: 134 - DNA, 17 bp, synthetic construct
  misc_feature 1..17: note = antisense oligonucleotides hybridizing with murine ANGPLT4
  source 1..17: mol_type = other DNA
agtactagactcgttag

SEQ ID NO: 135 - DNA, 17 bp, synthetic construct
  misc_feature 1..17: note = antisense oligonucleotides hybridizing with murine ANGPLT4
  source 1..17: mol_type = other DNA
tcggcaacctcctctta

SEQ ID NO: 136 - DNA, 17 bp, synthetic construct
  misc_feature 1..17: note = antisense oligonucleotides hybridizing with murine ANGPLT4
  source 1..17: mol_type = other DNA
gctttatgtcggcaacc

SEQ ID NO: 137 - DNA, 17 bp, synthetic construct
  misc_feature 1..17: note = antisense oligonucleotides hybridizing with murine ANGPLT4
  source 1..17: mol_type = other DNA
ttgactcatgccataac

SEQ ID NO: 138 - DNA, 17 bp, synthetic construct
  misc_feature 1..17: note = antisense oligonucleotides hybridizing with murine ANGPLT4
  source 1..17: mol_type = other DNA
gttaacggctaataaga

SEQ ID NO: 139 - DNA, 17 bp, synthetic construct
  misc_feature 1..17: note = antisense oligonucleotides hybridizing with murine ANGPLT4
  source 1..17: mol_type = other DNA
tctggttaacggctaat

SEQ ID NO: 140 - DNA, 17 bp, synthetic construct
  misc_feature 1..17: note = antisense oligonucleotides hybridizing with murine ANGPLT4
  source 1..17: mol_type = other DNA
actttagctccttatga

SEQ ID NO: 141 - DNA, 17 bp, synthetic construct
  misc_feature 1..17: note = antisense oligonucleotides hybridizing with murine ANGPLT4
  source 1..17: mol_type = other DNA
gatcgaaactgttatgt

SEQ ID NO: 142 - DNA, 17 bp, synthetic construct
  misc_feature 1..17: note = antisense oligonucleotides hybridizing with murine ANGPLT4
  source 1..17: mol_type = other DNA
tcctctcatccaatcgg

SEQ ID NO: 143 - DNA, 17 bp, synthetic construct
  misc_feature 1..17: note = antisense oligonucleotides hybridizing with murine ANGPLT4
  source 1..17: mol_type = other DNA
acggctatgtctgttac

SEQ ID NO: 144 - DNA, 17 bp, synthetic construct
  misc_feature 1..17: note = antisense oligonucleotides hybridizing with murine ANGPLT4
  source 1..17: mol_type = other DNA
ggacctgtaaccaccta

SEQ ID NO: 145 - DNA, 17 bp, synthetic construct
  misc_feature 1..17: note = antisense oligonucleotides hybridizing with murine ANGPLT4
  source 1..17: mol_type = other DNA
gtattgtcgctgatgaa

SEQ ID NO: 146 - DNA, 17 bp, synthetic construct
  misc_feature 1..17: note = antisense oligonucleotides hybridizing with murine ANGPLT4
  source 1..17: mol_type = other DNA
gatttgcctaaactcgt

SEQ ID NO: 147 - DNA, 17 bp, synthetic construct
  misc_feature 1..17: note = antisense oligonucleotides hybridizing with murine ANGPLT4
  source 1..17: mol_type = other DNA
gagcttgcgatgcctgt

SEQ ID NO: 148 - DNA, 17 bp, synthetic construct
  misc_feature 1..17: note = antisense oligonucleotides hybridizing with murine ANGPLT4
  source 1..17: mol_type = other DNA
gtagatgactaggcctg

SEQ ID NO: 149 - DNA, 17 bp, synthetic construct
  misc_feature 1..17: note = antisense oligonucleotides hybridizing with murine ANGPLT4
  source 1..17: mol_type = other DNA
tcaatggaagcgcttta

SEQ ID NO: 150 - DNA, 17 bp, synthetic construct
  misc_feature 1..17: note = antisense oligonucleotides hybridizing with murine ANGPLT4
  source 1..17: mol_type = other DNA
gtagcagacttgcacta

SEQ ID NO: 151 - DNA, 17 bp, synthetic construct
  misc_feature 1..17: note = antisense oligonucleotides hybridizing with murine ANGPLT4
  source 1..17: mol_type = other DNA
ctcatgttaggtaggtt

SEQ ID NO: 152 - DNA, 17 bp, synthetic construct
  misc_feature 1..17: note = antisense oligonucleotides hybridizing with murine ANGPLT4
  source 1..17: mol_type = other DNA
acgtggccaaagacaat

SEQ ID NO: 153 - DNA, 24 bp, synthetic construct
  misc_feature 1..24: note = positive control CpG oligonucleotide
  source 1..24: mol_type = other DNA
tcgtcgttttgtcgttttgtcgtt

SEQ ID NO: 154 - DNA, 16 bp, synthetic construct
  misc_feature 1..16: note = antisense oligonucleotide
  source 1..16: mol_type = other DNA
caccggagagcatcga

SEQ ID NO: 155 - DNA, 17 bp, synthetic construct
  misc_feature 1..17: note = antisense oligonucleotide
  source 1..17: mol_type = other DNA
cacggcatgtaaggaag

SEQ ID NO: 156 - DNA, 17 bp, synthetic construct
  misc_feature 1..17: note = antisense oligonucleotide
  source 1..17: mol_type = other DNA
acacacggcatgtaagg

SEQ ID NO: 157 - DNA, 17 bp, synthetic construct
  misc_feature 1..17: note = antisense oligonucleotide
  source 1..17: mol_type = other DNA
tagtctcgacagcaggt

SEQ ID NO: 158 - DNA, 17 bp, synthetic construct
  misc_feature 1..17: note = antisense oligonucleotide
  source 1..17: mol_type = other DNA
ggttcgagatgaacgga

SEQ ID NO: 159 - DNA, 16 bp, synthetic construct
  misc_feature 1..16: note = antisense oligonucleotide
  source 1..16: mol_type = other DNA
tcgagatgaacggaga

SEQ ID NO: 160 - DNA, 17 bp, synthetic construct
  misc_feature 1..17: note = antisense oligonucleotide
  source 1..17: mol_type = other DNA
tctgcatcggacacacg

SEQ ID NO: 161 - DNA, 17 bp, synthetic construct
  misc_feature 1..17: note = antisense oligonucleotide
  source 1..17: mol_type = other DNA
aacttagagaaccgcga

SEQ ID NO: 162 - DNA, 17 bp, synthetic construct
  misc_feature 1..17: note = antisense oligonucleotide
  source 1..17: mol_type = other DNA
gccgtgaacttagagaa

SEQ ID NO: 163 - DNA, 16 bp, synthetic construct
  misc_feature 1..16: note = antisense oligonucleotide
  source 1..16: mol_type = other DNA
ttagagaaccgcgagt

SEQ ID NO: 164 - DNA, 17 bp, synthetic construct
  misc_feature 1..17: note = antisense oligonucleotide
  source 1..17: mol_type = other DNA
tgaccaggaagacgctt

SEQ ID NO: 165 - DNA, 17 bp, synthetic construct
  misc_feature 1..17: note = antisense oligonucleotide
  source 1..17: mol_type = other DNA
tcgaaatgagtctgcac

SEQ ID NO: 166 - DNA, 17 bp, synthetic construct
  misc_feature 1..17: note = antisense oligonucleotide
  source 1..17: mol_type = other DNA
cgttgagcacgtctgga

SEQ ID NO: 167 - DNA, 16 bp, synthetic construct
  misc_feature 1..16: note = antisense oligonucleotide
  source 1..16: mol_type = other DNA
cgttgagcacgtctgg

SEQ ID NO: 168 - DNA, 17 bp, synthetic construct
  misc_feature 1..17: note = antisense oligonucleotide
  source 1..17: mol_type = other DNA
cacacgtccagttctca

SEQ ID NO: 169 - DNA, 17 bp, synthetic construct
  misc_feature 1..17: note = antisense oligonucleotide
  source 1..17: mol_type = other DNA
gcggatcggtcaggagt

SEQ ID NO: 170 - DNA, 17 bp, synthetic construct
  misc_feature 1..17: note = antisense oligonucleotide
  source 1..17: mol_type = other DNA
taccacacaccgtcctg

SEQ ID NO: 171 - DNA, 17 bp, synthetic construct
  misc_feature 1..17: note = antisense oligonucleotide
  source 1..17: mol_type = other DNA
ccttgtaccacacaccg

SEQ ID NO: 172 - DNA, 16 bp, synthetic construct
  misc_feature 1..16: note = antisense oligonucleotide
  source 1..16: mol_type = other DNA
ttgtaccacacaccgt

SEQ ID NO: 173 - DNA, 17 bp, synthetic construct
  misc_feature 1..17: note = antisense oligonucleotide
  source 1..17: mol_type = other DNA
cttaacagtggatgacc

SEQ ID NO: 174 - DNA, 16 bp, synthetic construct
  misc_feature 1..16: note = antisense oligonucleotide
  source 1..16: mol_type = other DNA
cgaggacggtttttat

SEQ ID NO: 175 - DNA, 17 bp, synthetic construct
  misc_feature 1..17: note = antisense oligonucleotide
  source 1..17: mol_type = other DNA
aggatccgctcagctcg

SEQ ID NO: 176 - DNA, 17 bp, synthetic construct
  misc_feature 1..17: note = antisense oligonucleotide
  source 1..17: mol_type = other DNA
tcgtgtgaggatccgct

SEQ ID NO: 177 - DNA, 17 bp, synthetic construct
  misc_feature 1..17: note = antisense oligonucleotide
  source 1..17: mol_type = other DNA
aatcggatcacagtcgt

SEQ ID NO: 178 - DNA, 17 bp, synthetic construct
  misc_feature 1..17: note = antisense oligonucleotide
  source 1..17: mol_type = other DNA
tagcacggcggtggcgg

SEQ ID NO: 179 - DNA, 16 bp, synthetic construct
  misc_feature 1..16: note = antisense oligonucleotide
  source 1..16: mol_type = other DNA
tagcacggcggtggcg

SEQ ID NO: 180 - DNA, 16 bp, synthetic construct
  misc_feature 1..16: note = antisense oligonucleotide
  source 1..16: mol_type = other DNA
gcggcgacttggactg

SEQ ID NO: 181 - DNA, 16 bp, synthetic construct
  misc_feature 1..16: note = antisense oligonucleotide
  source 1..16: mol_type = other DNA
ggacgcaaagcgcggc

SEQ ID NO: 182 - DNA, 16 bp, synthetic construct
  misc_feature 1..16: note = antisense oligonucleotide
  source 1..16: mol_type = other DNA
aggacgcaaagcgcgg

SEQ ID NO: 183 - DNA, 17 bp, synthetic construct
  misc_feature 1..17: note = antisense oligonucleotide
  source 1..17: mol_type = other DNA
gcggctgacattgtgag

SEQ ID NO: 184 - DNA, 17 bp, synthetic construct
  misc_feature 1..17: note = antisense oligonucleotide
  source 1..17: mol_type = other DNA
ataggccgtgtcctcgc

SEQ ID NO: 185 - DNA, 17 bp, synthetic construct
  misc_feature 1..17: note = antisense oligonucleotide
  source 1..17: mol_type = other DNA
tataggccgtgtcctcg

SEQ ID NO: 186 - DNA, 17 bp, synthetic construct
  misc_feature 1..17: note = antisense oligonucleotide
  source 1..17: mol_type = other DNA
agtactggccgttgagg

SEQ ID NO: 187 - DNA, 17 bp, synthetic construct
  misc_feature 1..17: note = antisense oligonucleotide
  source 1..17: mol_type = other DNA
gaagtactggccgttga

SEQ ID NO: 188 - DNA, 17 bp, synthetic construct
  misc_feature 1..17: note = antisense oligonucleotide
  source 1..17: mol_type = other DNA
tcttaagcttctgccgc

SEQ ID NO: 189 - DNA, 17 bp, synthetic construct
  misc_feature 1..17: note = antisense oligonucleotide
  source 1..17: mol_type = other DNA
agtcaccgtctttcgtg

SEQ ID NO: 190 - DNA, 17 bp, synthetic construct
  misc_feature 1..17: note = antisense oligonucleotide
  source 1..17: mol_type = other DNA
cgccattgaggccagtc

SEQ ID NO: 191 - DNA, 17 bp, synthetic construct
  misc_feature 1..17: note = antisense oligonucleotide
  source 1..17: mol_type = other DNA
ctgagtccgccattgag

SEQ ID NO: 192 - DNA, 17 bp, synthetic construct
  misc_feature 1..17: note = antisense oligonucleotide
  source 1..17: mol_type = other DNA
attggcgcctgcttgtg

SEQ ID NO: 193 - DNA, 17 bp, synthetic construct
  misc_feature 1..17: note = antisense oligonucleotide
  source 1..17: mol_type = other DNA
ataccattggcgcctgc

SEQ ID NO: 194 - DNA, 17 bp, synthetic construct
  misc_feature 1..17: note = antisense oligonucleotide
  source 1..17: mol_type = other DNA
tgagtccgccattgagg

SEQ ID NO: 195 - DNA, 17 bp, synthetic construct
  misc_feature 1..17: note = antisense oligonucleotide
  source 1..17: mol_type = other DNA
actgagtccgccattga

SEQ ID NO: 196 - DNA, 17 bp, synthetic construct
  misc_feature 1..17: note = antisense oligonucleotide
  source 1..17: mol_type = other DNA
tgactgagtccgccatt

SEQ ID NO: 197 - DNA, 17 bp, synthetic construct
  misc_feature 1..17: note = antisense oligonucleotide
  source 1..17: mol_type = other DNA
tgtgactgagtccgcca

SEQ ID NO: 198 - DNA, 17 bp, synthetic construct
  misc_feature 1..17: note = antisense oligonucleotide
  source 1..17: mol_type = other DNA
ccccgtcagtcaatgtg

SEQ ID NO: 199 - DNA, 17 bp, synthetic construct
  misc_feature 1..17: note = antisense oligonucleotide
  source 1..17: mol_type = other DNA
ggtccccgtcagtcaat

SEQ ID NO: 200 - DNA, 17 bp, synthetic construct
  misc_feature 1..17: note = antisense oligonucleotide
  source 1..17: mol_type = other DNA
ttcacggttgcacctaa

SEQ ID NO: 201 - DNA, 16 bp, synthetic construct
  misc_feature 1..16: note = antisense oligonucleotide
  source 1..16: mol_type = other DNA
ataagcgtttcacggt

SEQ ID NO: 202 - DNA, 17 bp, synthetic construct
  misc_feature 1..17: note = antisense oligonucleotide
  source 1..17: mol_type = other DNA
gctaggactccggaacg

SEQ ID NO: 203 - DNA, 17 bp, synthetic construct
  misc_feature 1..17: note = antisense oligonucleotide
  source 1..17: mol_type = other DNA
cagcaacgctaggactc

SEQ ID NO: 204 - DNA, 17 bp, synthetic construct
  misc_feature 1..17: note = antisense oligonucleotide
  source 1..17: mol_type = other DNA
gtgcagcaacgctagga

SEQ ID NO: 205 - DNA, 17 bp, synthetic construct
  misc_feature 1..17: note = antisense oligonucleotide
  source 1..17: mol_type = other DNA
ccgcgcatagcaccagg

SEQ ID NO: 206 - DNA, 17 bp, synthetic construct
  misc_feature 1..17: note = antisense oligonucleotide
  source 1..17: mol_type = other DNA
atgcaaagcgcggtggc

SEQ ID NO: 207 - DNA, 17 bp, synthetic construct
  misc_feature 1..17: note = antisense oligonucleotide
  source 1..17: mol_type = other DNA
ccacgtgttcgcgcagc

SEQ ID NO: 208 - DNA, 17 bp, synthetic construct
  misc_feature 1..17: note = antisense oligonucleotide
  source 1..17: mol_type = other DNA
agcgttaccacaggcag

SEQ ID NO: 209 - DNA, 17 bp, synthetic construct
  misc_feature 1..17: note = antisense oligonucleotide
  source 1..17: mol_type = other DNA
tctatcctcggagtctt

SEQ ID NO: 210 - DNA, 17 bp, synthetic construct
  misc_feature 1..17: note = antisense oligonucleotide
  source 1..17: mol_type = other DNA
ctcgaagtcttgtctac

SEQ ID NO: 211 - DNA, 17 bp, synthetic construct
  misc_feature 1..17: note = antisense oligonucleotide
  source 1..17: mol_type = other DNA
gaagtattgtccattga

SEQ ID NO: 212 - DNA, 17 bp, synthetic construct
  misc_feature 1..17: note = antisense oligonucleotide
  source 1..17: mol_type = other DNA
cagaggatagtagcggc

SEQ ID NO: 213 - DNA, 17 bp, synthetic construct
  misc_feature 1..17: note = antisense oligonucleotide
  source 1..17: mol_type = other DNA
cagtctctccagttacg

SEQ ID NO: 214 - DNA, 16 bp, synthetic construct
  misc_feature 1..16: note = antisense oligonucleotide
  source 1..16: mol_type = other DNA
gcgagaagtgatattc

SEQ ID NO: 215 - DNA, 17 bp, synthetic construct
  misc_feature 1..17: note = antisense oligonucleotide
  source 1..17: mol_type = other DNA
tcaatatgactgagtcc

SEQ ID NO: 216 - DNA, 17 bp, synthetic construct
  misc_feature 1..17: note = antisense oligonucleotide
  source 1..17: mol_type = other DNA
tccagtcagtcaatatg

SEQ ID NO: 217 - DNA, 17 bp, synthetic construct
  misc_feature 1..17: note = antisense oligonucleotide
  source 1..17: mol_type = other DNA
ctccagtcagtcaatat

SEQ ID NO: 218 - DNA, 17 bp, synthetic construct
  misc_feature 1..17: note = antisense oligonucleotide
  source 1..17: mol_type = other DNA
gagtcctagtagatgcg

SEQ ID NO: 219 - DNA, 17 bp, synthetic construct
  misc_feature 1..17: note = antisense oligonucleotide
  source 1..17: mol_type = other DNA
gttagtctaagtagagt

SEQ ID NO: 220 - DNA, 16 bp, synthetic construct
  misc_feature 1..16: note = antisense oligonucleotide
  source 1..16: mol_type = other DNA
agtactagactcgtta

SEQ ID NO: 221 - DNA, 17 bp, synthetic construct
  misc_feature 1..17: note = antisense oligonucleotide
  source 1..17: mol_type = other DNA
gcaacctcctcttattc

SEQ ID NO: 222 - DNA, 17 bp, synthetic construct
  misc_feature 1..17: note = antisense oligonucleotide
  source 1..17: mol_type = other DNA
aagatatgcaaggctag

SEQ ID NO: 223 - DNA, 17 bp, synthetic construct
  misc_feature 1..17: note = antisense oligonucleotide
  source 1..17: mol_type = other DNA
gactcatgccataacaa

SEQ ID NO: 224 - DNA, 17 bp, synthetic construct
  misc_feature 1..17: note = antisense oligonucleotide
  source 1..17: mol_type = other DNA
gtggacctgacaagaag

SEQ ID NO: 225 - DNA, 17 bp, synthetic construct
  misc_feature 1..17: note = antisense oligonucleotide
  source 1..17: mol_type = other DNA
aacggctaataagattt

SEQ ID NO: 226 - DNA, 17 bp, synthetic construct
  misc_feature 1..17: note = antisense oligonucleotide
  source 1..17: mol_type = other DNA
gttctggttaacggcta

SEQ ID NO: 227 - DNA, 17 bp, synthetic construct
  misc_feature 1..17: note = antisense oligonucleotide
  source 1..17: mol_type = other DNA
ggtgtgcttactctggt

SEQ ID NO: 228 - DNA, 17 bp, synthetic construct
  misc_feature 1..17: note = antisense oligonucleotide
  source 1..17: mol_type = other DNA
cctagaaattgtgatcg

SEQ ID NO: 229 - DNA, 17 bp, synthetic construct
  misc_feature 1..17: note = antisense oligonucleotide
  source 1..17: mol_type = other DNA
aacgaataggcatgaac

SEQ ID NO: 230 - DNA, 17 bp, synthetic construct
  misc_feature 1..17: note = antisense oligonucleotide
  source 1..17: mol_type = other DNA
actttcacctagttggc

SEQ ID NO: 231 - DNA, 17 bp, synthetic construct
  misc_feature 1..17: note = antisense oligonucleotide
  source 1..17: mol_type = other DNA
ctctacttggctaggct

SEQ ID NO: 232 - DNA, 17 bp, synthetic construct
  misc_feature 1..17: note = antisense oligonucleotide
  source 1..17: mol_type = other DNA
ggtactctgaattagta

SEQ ID NO: 233 - DNA, 17 bp, synthetic construct
  misc_feature 1..17: note = antisense oligonucleotide
  source 1..17: mol_type = other DNA
tgtaaccacctaaagcc

SEQ ID NO: 234 - DNA, 17 bp, synthetic construct
  misc_feature 1..17: note = antisense oligonucleotide
  source 1..17: mol_type = other DNA
aggtattgtcgctgatg

SEQ ID NO: 235 - DNA, 17 bp, synthetic construct
  misc_feature 1..17: note = antisense oligonucleotide
  source 1..17: mol_type = other DNA
gaacagaggtattgtcg

SEQ ID NO: 236 - DNA, 17 bp, synthetic construct
  misc_feature 1..17: note = antisense oligonucleotide
  source 1..17: mol_type = other DNA
catgtatcacaccttcc

SEQ ID NO: 237 - DNA, 17 bp, synthetic construct
  misc_feature 1..17: note = antisense oligonucleotide
  source 1..17: mol_type = other DNA
taaactcgttcctgcct

SEQ ID NO: 238 - DNA, 17 bp, synthetic construct
  misc_feature 1..17: note = antisense oligonucleotide
  source 1..17: mol_type = other DNA
gcctaaactcgttcctg

SEQ ID NO: 239 - DNA, 17 bp, synthetic construct
  misc_feature 1..17: note = antisense oligonucleotide
  source 1..17: mol_type = other DNA
atctcaggagcttatac

SEQ ID NO: 240 - DNA, 17 bp, synthetic construct
  misc_feature 1..17: note = antisense oligonucleotide
  source 1..17: mol_type = other DNA
acaagctgcataatagg

SEQ ID NO: 241 - DNA, 17 bp, synthetic construct
  misc_feature 1..17: note = antisense oligonucleotide
  source 1..17: mol_type = other DNA
tatcactgagcttgcga

SEQ ID NO: 242 - DNA, 17 bp, synthetic construct
  misc_feature 1..17: note = antisense oligonucleotide
  source 1..17: mol_type = other DNA
aatggaagcgctttacc

SEQ ID NO: 243 - DNA, 17 bp, synthetic construct
  misc_feature 1..17: note = antisense oligonucleotide
  source 1..17: mol_type = other DNA
tagcagacttgcactat

SEQ ID NO: 244 - DNA, 17 bp, synthetic construct
  misc_feature 1..17: note = antisense oligonucleotide
  source 1..17: mol_type = other DNA
aggctcaactctcgcac

SEQ ID NO: 245 - DNA, 17 bp, synthetic construct
  misc_feature 1..17: note = antisense oligonucleotide
  source 1..17: mol_type = other DNA
aagagctagtactgtag

SEQ ID NO: 246 - DNA, 17 bp, synthetic construct
  misc_feature 1..17: note = antisense oligonucleotide
  source 1..17: mol_type = other DNA
tataatttgatcctgac

SEQ ID NO: 247 - DNA, 17 bp, synthetic construct
  misc_feature 1..17: note = antisense oligonucleotide
  source 1..17: mol_type = other DNA
ggttctctgccaaatga

SEQ ID NO: 248 - DNA, 17 bp, synthetic construct
  misc_feature 1..17: note = antisense oligonucleotide
  source 1..17: mol_type = other DNA
cgtggccaaagacaatt

SEQ ID NO: 249 - DNA, 16 bp, synthetic construct
  misc_feature 1..16: note = Negative control oligonucleotide
  source 1..16: mol_type = other DNA
tacgcgcggttgttta

SEQ ID NO: 250 - DNA, 16 bp, synthetic construct
  misc_feature 1..16: note = Negative control oligonucleotide
  source 1..16: mol_type = other DNA
ttagcgcgcgaatatg

SEQ ID NO: 251 - DNA, 17 bp, synthetic construct
  misc_feature 1..17: note = Negative control oligonucleotide
  source 1..17: mol_type = other DNA
cgaataaccgtcgtgtt

SEQ ID NO: 252 - DNA, 17 bp, synthetic construct
  misc_feature 1..17: note = Negative control oligonucleotide
  source 1..17: mol_type = other DNA
gactcgttaaaccgata